European Patent Specification EP 3 110 441 B1, published April 3, 2024. Title: NOVEL POLYSACCHARIDE AND USES THEREOF. Applicant: GlycoVaxyn AG. Application TBA. The sequence listing filed with the application follows.

SEQUENCE LISTING (15 sequences)

SEQ ID NO: 1 - DNA, 1086 bp, E. Coli
  rmlB (upec138)
gtgaagatacttgttactggtggcgcaggatttattggttctgctgttgttcgtcacataataaataatacgcaagatagtgttgttaatgtcgataaattaacatacgccggaaacctggaatcacttgcagatgtttctgattctgaacgctatttctttgaacatgcggatatttgtgatgcagctgcaatggcacggatttttgctcagcatcagccggatgcagtgatgcacctggcagctgaaagccatgttgaccgttcaattacaggccctgcggcatttattgaaaccaatattgtgggtacttatgtccttttagaagcggctcggaattattggtctggtctggatgatgaaaagaaaaaaaacttccgttttcatcatatttctactgatgaggtgtatggtgacttaccccatccggatgaagtaaatagcaatgaaacgttgccgctatttacggaaacgacagcatacgcgccaagtagtccatattctgcttctaaagcttccagcgatcatttggttcgcgcatggaaacgtacttatggtttaccgaccattgtgactaattgctcgaacaactatggtccttatcatttcccggaaaagcttattccactggttattcttaattcactggaaggtaaggcattacctatttatggcaaaggagatcagatccgcgactggttgtatgtagaggatcatgctcgagcgttatataccgtcgtaaccgaaggtaaagcgggcgaaacttataacattggtggacacaacgaaaagaaaaacatcgacgtagtgttcactatttgtgatttgttggatgagatagtcccgaaagagaaatcttaccgcgagcaaattacttatgttaccgatcgtccgggacacgatcgccgttatgcgattgatgctgagaagattggtcgcgaattgggatggaaaccacaggaaacgtttgagagtgggattcgtaaaacggtggaatggtacctgtccaatacaaaatgggttgataatgtgaaaagtggtgcctatcaatcgtggattgaacagaactatgagggccgccagtaa

SEQ ID NO: 2 - DNA, 900 bp, E. Coli
  rmlD (upec138)
atgaatatcctcctttttggcaaaacagggcaggtaggttgggaactacagcgtgctctggcacctctgggtaatttgattgctcttgatgttcactccactgattactgtggtgattttagtaatcctgaaggtgtagctgaaaccgtaagaagcattcggcctgatattattgtcaacgcagccgctcacaccgcagtagacaaagcagaatcagaaccgaagtttgcacaattactgaacgcgacgagtgtcgaagcgatcgcgaaagcagccaatgaagtcggcgcctgggttattcactactctactgactacgtatttccggggaccggtgaaataccatggcaggaggaggatgcaaccgcaccgctaaatgtttacggtgaaaccaagttagcgggagaaaaagcattacaagagcattgtgcgaagcaccttattttccggaccagctgggtctatgcaggtaaaggaaataacttcgccaaaacaatgttgcgtctggcaaaagagcgtgaagaattagccgttattaatgatcagtttggtgcgccaactggcgcagagttactggctgattgtacggcacatgctattcgtgtggcactgaataaaccggaagtcgcaggcttgtaccatctggtagctagtggtaccacaacgtggcacgattatgctgcgctggtttttgaagaggcgcgcaaagcaggcattccccttgcactcaacaagctcaacgcagtaccaacaacagcctatcctacaccagctcgtcgtccacataactctcgccttaatacagaaaaatttcagcagaactttgcgcttgtcttgcctgactggcaggttggcgtgaaacgaatgcttaacgaattatttacgactacagcaatttaa

SEQ ID NO: 3 - DNA, 879 bp, E. Coli
  rmlA (upec138)
atgaaaacgcgtaaaggtattattttggcgggtggttctggtactcgtctttatcctgtgacgatggccgtcagtaaacagctgttaccgatttatgataaaccgatgatctattacccgctctctacactgatgttagcgggtattcgcgatattctgattatcagtacaccacaggatactcctcgttttcaacaactgctgggtgacgggagccagtggggcctgaatcttcagtacaaagtgcaaccgagtccggatggtcttgcgcaggcgtttattatcggtgaagagtttattggtggtgatgattgtgctttggtacttggtgataatatcttctacggccacgacctgccgaagttaatggacgtagctgttaacaaagaaagtggtgcaacggtatttgcctatcacgttaatgatcctgaacgttatggtgtcgtggagtttgataataacggtactgcaattagcctggaagaaaaaccgctggaaccaaaaagtaactatgcggttactgggctttatttctatgacaatgacgttgtggaaatggcgaaaaaccttaagccttctgcccgaggtgaactggaaattaccgatattaaccgtatttatatggaacaaggacgtttgtctgtcgctatgatggggcgtggctatgcatggctggatacagggacgcatcaaagtcttattgaagcaagcaacttcattgccaccattgaagagcgccagggactaaaggtttcctgtccggaagaaattgcttatcgtaaagggtttattgatgctgagcaggtaaaagtattagccgaaccgttgaagaaaaatgcttatggtcagtatctgctcaaaatgattaaaggttattaa

SEQ ID NO: 4 - DNA, 543 bp, E. Coli
  rmlC (upec138)
atgaacgtaattaaaactgaaattcctgatgtgctgatttttgaaccaaaagtttttggggatgaacgtggcttcttttttgagagttttaatcagaggatttttgaagaagcagtaggtcgtaaggttgagtttgttcaggataaccattctaagtccagtaaaggtgttttacgtggtcttcattatcagttagaaccttatgctcaaggaaaactggtgcgctgtgttgttggcgaggtttttgatgttgcggttgatattcgtaaatcgtcacctacatttgggaaatgggttggggtgaatttgtctgctgagaataagcgtcagttgtggattcctgagggatttgcacatggttttttggtgctgagtgatttagcagaagttttatataaaacgaatcaatattatgctccatcacatgaaaaaaatattatatggaatgacctcttgcttaatattaaatggccgagcacagcactgatcactctgtctgataaggatgcaaatggggaaagatttgaactaagtgagttttga

SEQ ID NO: 5 - DNA, 1260 bp, E. Coli
  wzx (upec138)
atgtctctcttaaaacatagtatatggaatgttgcgggctactttataccaacattaattgcaattcccgcctttggattaattgcgaggaaaattggtgtagaactatttggtttgtatacgttagcaatgatttttatagggtatgcaagtatatttgatgctgggttaacaagagctgttgtgcgtgaaatagcattactaaaaaacagagtggacgattgtaatacgataatagtaacttctattatcgctgtgatatttttagggtttatcggaggcgggggagtgtttctgcttaaaggcgatattattgaactgttaaatatctcaccaatatattacgccgattcgataaagtctctagtattattatcatctctgatacctgtattcttagtcacgcaaatactattagcagagcttgagggtcgggaatattttgggattctaaatatacaaaaaagtgtagggaattctttaattgcagggttacctgcattatttgttttaattaatcaaacgcttttttctgcaattattggtgtagcgattgcaagagttatatgcttgtggttaagctacattatgagcagggaaagaataactatcgatatctcatttttttcaataactgttttaaagcggttatttagatatggcgggtgggtaactataagtaacataatatctcctatattagcgagtatggatagatttattctatcccatatccagggagcatcaaaaatatcattctatacagtccctaatgagctggtaactaggcttggaatagttccaggctctcttgggaaagctgtttttccaaaattaagtcatgcaaggaattttacagcgtcatatgcagagcaaaaaaaagcttatatattaatgactgtcattgtaatgcctttggttttatttgtatattattacgcaaagtttattttaacattgtggatgggggctgagtatgcagggatttcggtcgaaatattacggattatgcttatagggtatatttttaactgttattcacaaatctcttttgccaacatacaggcctttggaaaagcaaaatacactgcatacatccatatgatggaatttattccttatttgataatgttatatataatttcaaaggaatatggggttattggtgttgcgtggttatggacaattcgagtaataattgattttttgatgcttttatatatgagttatcgttgtaataatcttatgaaaaaagggtag

SEQ ID NO: 6 - DNA, 966 bp, E. Coli
  wekA (upec138)
atgatatatattgtggtattaaattggaatggggctatagataccattaattgtgttaaaagtttaatggatttaaatgttagcgattataaaattatcattgttgataactgttctatggataactcatatgatactataaaagaaaatcttaattcattatatattgctgataaaagtatcattgaggtgaagtatgaggatagaaataaatataaaaccttagaaaacgataaaatcatattaatacaatctccgcaaaataatgggtacgcaagtggtaataatattggcatagagttcgctcttaatcaggagaatatgaaatacgtctgggttctgaataatgatactgaagtggataaagaggctttaactcatttaattagtaaatgtgattcagataaaagtatagggatttgcggttctcgtttagtctattttgccgacagagagatgcagcaaggactaggtggggtgcataacaaatggttatgcactacaaaaaattatgaaatgggaagattagtttccaaaaaatatgatgatgaagtcattagtaatgatatagattatataattggcgcatcgatgtttttctctagagaatgtttggaaacagttggattgatgaatgaagaatattttttatactatgaagagttagatatttgcctcagagcaaaagcaaagaactttaaattaggtatttgctcagaaagtttggtttatcataaaataggtgcaagtactgatgggggaaagagcatgatggctgatctttgctcaataaaaaataggctggtcattacagaaaggttttatccccaatattattggacggtatggttgtcactttttgttgtagcatttaaccgtgctagaagaggtgagtttaataagatgaaaagatgtttgaatgttatgtttaacttcaaacgaaacaaaggtagcaaatgccattag

SEQ ID NO: 7 - DNA, 1149 bp, E. Coli
  wekB (upec138)
atgaaagtggcttttttatctgcttatgatccactatctacatccagttggtctggcacaccttattatatgctaaaggcattatcgaagagaaatatttccattgaaatattaggaccggtaaatagctatatgatatacatgttaaaagtatataaattaatattaaggtgtttcggaaaagaatatgattatagtcattcgaagttgctttccaggtattacggtagaatattcggtaggaaattaaaaaaaattgatggtttggattttattatcgcacctgcaggttcctcacaaattgcttttttaaaaacaaccataccaataatatatctatcggatacaacatatgatcaattaaaaagctattatccgaatttaaataaaaaaacaattataaatgatgaggatgcaagtttaatcgaacgcaaggctattgaaaaagcaacagtagtatctttcccatctaaatgggcaatggatttttgcaggaattattacagattagattttgataaattagttgaaataccatggggggctaatttatttgatgatattcactttgctaataaaaatataattcaaaagaatagttatacttgtcttttcttgggagttgattgggaaagaaaaggtgggaaaacagccttgaaagcaattgaatatgtaaggcagttatatgggatcgatgttagactaaaaatttgtggatgtactccgaatcaaaagattttacctacttgggttgaattaattgataaagtagataaaaataacgttgacgaatatcagaaattcatcgatgtgttatctaacgctgatatacttcttttaccaaccattgctgaatgttatggaatggtattttgtgaagctgctgcttttggattgcctgttgtcgctacagatacaggtggagtcagttctatagttatcaacgaaaggacggggatattaattaaagacccgttagactataagcactttggaaatgcaattcataaaataattagttccgtagagacttatcaaaactactcccaaaacgcaagaattagatataataatatattgcattgggacaattgggctaaaaagataattgagattatgtatgagcataagaatagaagaatcaaatag

SEQ ID NO: 8 - DNA, 1218 bp, E. Coli
  wzy (upec138)
atgagcataagaatagaagaatcaaatagcacaaaaagaattatatgtttatttatactttttcttgttttccctgattttttgttttatacattaggggttgataattttagcatttcaacgataatctcaattacattgctttttgtttttttaagagctaaaaatatttgcaaagataattttctaataatagtagcgttattcatattgttgtgttttaactgtttgttaagtatgctatttaatattgaacaggctttaacatttaaagttgtactttcaatatatagcatcttaataatggcatacgtctcctcttgttatgcacagacgttgtggttatgttctgaagaaatacttaagagatccgtcttttatttgttcgcatttctttgccttattggcattataagtattcttttacagaagactgagattatacatgataaaagtatgattctttttcctgaaccatcagcatttgcattggtttttatacctatcttttcattttgtttatactatacaagagggggggggctactattgctctatatattatctttgggtattgcgttaggtatccagaatttaacaatgttggtaggcattgtgattagtgtttttgtgatgaaaaaaataactataaggcaaactattgttatacttttgggggcatggattttttccatgatattaagtgatttagacatttcttactatacatcgcggcttgattttaaaaatactacgaacctatcagtgcttgtatatctttcaggaattgaaagagctttcttgaattttattacaagttatggtcttggtattggttttcaacaaatgggagtgaatggggagataggaatatatcaacaaattttagctgaacttgatgcccctatgttaaatatatacgatggctcatttatttcttctaagttaatatctgagtttggggttattggtgcattaatgtgtattttctattttttttatttttcccgattttatctgcgtttcaaaaaaagtaagagatattcaccgcagtatattttagcatatagcttctacatgtgtttcttcatccctctttttatacgtggtgctggttatataaacccctatgtgtttatgttattttcatcaatatttttgtgcaaatatcacgctaaaaatatcttgatgaaatctaatgtccagatagctatataa

SEQ ID NO: 9 - DNA, 606 bp, E. Coli
  wbbJ (upec138)
atgtgcattaaaaaaaaacttaagttaattaaacgatatggcctttatggtggtcttaggcttcttaaagatatattcttaacaaaatttttattttgttcaaatgttaggattattagatttccatgttatattagaaaagatggaagtgttagttttggaaaaggttttacatcaggtgtaggattacgagttgatgcatttatggatgccgtagtttccattggagaaaatgttcaaattaatgactatgttcacatcgcggctattaataatgtcattattggtagagatacattaatagcaagtaaagtatttattagtgatcataatcatggtattttttctaaatccgatatccatagttcaccaactattattccttcgtctaggccccttgaatctgcacctgtgtatattggagagcgtgtgtggattggcgaaaatgtgacaatattaccaggtgcgtgtataggtaatggtgtagttattggcgcaaacagtgttgttcgtggtgagattcctaataatgtgatcattgctggtgttccagctaaaattgttaaaaaatataactatgagcgtatgcaatgggaaagaatatag

SEQ ID NO: 10 - DNA, 1101 bp, E. Coli
  wbbK (upec138)
atgggaaagaatatagttgtaatatcggctgttaattttacaaccggaggcccctttaccgtactaaaaaatgtgcttacagcaactaaagatagagccgaatgtaaatttattgcactggttcatagctctgctgaactaatggaattatttccgtgggttgaatttatagagtatccagaagtcaagtcttcgtgggttaaaagattatatttcgaatatataacttgcaatagattatctaaggtgattaaggcaactcattgggtatgcttacatgatattacagcaaatgttagtgtaccctatagatttgtttattgccacaatcctgcaccgttctataaatatttaagctatcgagatattataggagaacctaaattttatcttttttatcttttttatgggcttttatacaatatcaatataaaaaagaacacagcagtttttgttcagcagcagtggctaaaaaaagaattcgaaaaaaaatataagttaaagaatgttgttgttagtcgccctgaagatatttgcccttttgaaagtgatggtttggtaagaaataataataaaaaggatgtgaggatattttacccagcagtgccccgtatatttaaaaactttgaagttatcatacgtgctgcacaaatattacaagataaaaatattcatttttatcttacttttgatggtactgaaaataagtatgcaaaaagaatatataaattagcttccgaactgaaaaatgtacatttcctcggttaccttaatgcaaccgagatggttaacttttatcaagattcagatattatttgtttcccatcgaaactagaaacgtggggattaccattatcagaagctaaaacatacaaaaaatggatatttgcggcagacttaccttatgctcatgaagttttatataactattcaaaaactagatattttccatttgacgatgagaaaatacttgttcgctacatattagagtacacaagtaaaaatatgcatgaagatataaaaaatagtagggtgaattttaataatgatgcattgactggttttgaacagtttattgaatatatcctcaaggggaactga

SEQ ID NO: 11 - DNA, 564 bp, E. Coli
  wbbL (upec138)
atgattatgaataatgattattttctctttcttaaccccgatgtattcataaccagtgaaagtttgattaattatgttgattatataattagtaatgattataagtttagcacattatgtctttatcgagattttactaaaagcaaacatgattattcaatacggagttttccaactttatatgattttctttgttcttttttattgggggtgaataaaagtaaaattaagaaggaaaatatactttctgatactgtagttgattggtgtgctggctcatttatgcttattcatgctttaagtttcttaaatgtgaatggttttgatcaaaaatattttatgtattgtgaagatattgacctttgtatgcgtttaaaattaagtggagtagatctttactatactccccattttgatgctattcattatgcgcagcatgaaaatagaagaatatttactaaagcatttcgatggcatataaggagtattacgcgctacatattacggaaaccaattctttcttataaaaactatagaaaaattacatccgaactggtaaagtga

SEQ ID NO: 12 - DNA, 10653 bp, E. Coli
  E. coli rfb(upec138) gene cluster
gtgaagatacttgttactggtggcgcaggatttattggttctgctgttgttcgtcacataataaataatacgcaagatagtgttgttaatgtcgataaattaacatacgccggaaacctggaatcacttgcagatgtttctgattctgaacgctatttctttgaacatgcggatatttgtgatgcagctgcaatggcacggatttttgctcagcatcagccggatgcagtgatgcacctggcagctgaaagccatgttgaccgttcaattacaggccctgcggcatttattgaaaccaatattgtgggtacttatgtccttttagaagcggctcggaattattggtctggtctggatgatgaaaagaaaaaaaacttccgttttcatcatatttctactgatgaggtgtatggtgacttaccccatccggatgaagtaaatagcaatgaaacgttgccgctatttacggaaacgacagcatacgcgccaagtagtccatattctgcttctaaagcttccagcgatcatttggttcgcgcatggaaacgtacttatggtttaccgaccattgtgactaattgctcgaacaactatggtccttatcatttcccggaaaagcttattccactggttattcttaattcactggaaggtaaggcattacctatttatggcaaaggagatcagatccgcgactggttgtatgtagaggatcatgctcgagcgttatataccgtcgtaaccgaaggtaaagcgggcgaaacttataacattggtggacacaacgaaaagaaaaacatcgacgtagtgttcactatttgtgatttgttggatgagatagtcccgaaagagaaatcttaccgcgagcaaattacttatgttaccgatcgtccgggacacgatcgccgttatgcgattgatgctgagaagattggtcgcgaattgggatggaaaccacaggaaacgtttgagagtgggattcgtaaaacggtggaatggtacctgtccaatacaaaatgggttgataatgtgaaaagtggtgcctatcaatcgtggattgaacagaactatgagggccgccagtaatgaatatcctcctttttggcaaaacagggcaggtaggttgggaactacagcgtgctctggcacctctgggtaatttgattgctcttgatgttcactccactgattactgtggtgattttagtaatcctgaaggtgtagctgaaaccgtaagaagcattcggcctgatattattgtcaacgcagccgctcacaccgcagtagacaaagcagaatcagaaccgaagtttgcacaattactgaacgcgacgagtgtcgaagcgatcgcgaaagcagccaatgaagtcggcgcctgggttattcactactctactgactacgtatttccggggaccggtgaaataccatggcaggaggaggatgcaaccgcaccgctaaatgtttacggtgaaaccaagttagcgggagaaaaagcattacaagagcattgtgcgaagcaccttattttccggaccagctgggtctatgcaggtaaaggaaataacttcgccaaaacaatgttgcgtctggcaaaagagcgtgaagaattagccgttattaatgatcagtttggtgcgccaactggcgcagagttactggctgattgtacggcacatgctattcgtgtggcactgaataaaccggaagtcgcaggcttgtaccatctggtagctagtggtaccacaacgtggcacgattatgctgcgctggtttttgaagaggcgcgcaaagcaggcattccccttgcactcaacaagctcaacgcagtaccaacaacagcctatcctacaccagctcgtcgtccacataactctcgccttaatacagaaaaatttcagcagaactttgcgcttgtcttgcctgactggcaggttggcgtgaaacgaatgcttaacgaattatttacgactacagcaatttaatagtttttgcatcttgttcgtaatggtggagcaagatgtattaaaaggaatgatgaaatgaaaacgcgtaaaggtattattttggcgggtggttctggtactcgtctttatcctgtgacgatggccgtcagtaaacagctgttaccgatttatgataaaccgatgatctattacccgctctctacactgatgttagcgggtattcgcgatattctgattatcagtacaccacaggatactcctcgttttcaacaactgctgggtgacgggagccagtggggcctgaatcttcagtacaaagtgcaaccgagtccggatggtcttgcgcaggcgtttattatcggtgaagagtttattggtggtgatgattgtgctttggtacttggtgataatatcttctacggccacgacctgccgaagttaatggacgtagctgttaacaaagaaagtggtgcaacggtatttgcctatcacgttaatgatcctgaacgttatggtgtcgtggagtttgataataacggtactgcaattagcctggaagaaaaaccgctggaaccaaaaagtaactatgcggttactgggctttatttctatgacaatgacgttgtggaaatggcgaaaaaccttaagccttctgcccgaggtgaactggaaattaccgatattaaccgtatttatatggaacaaggacgtttgtctgtcgctatgatggggcgtggctatgcatggctggatacagggacgcatcaaagtcttattgaagcaagcaacttcattgccaccattgaagagcgccagggactaaaggtttcctgtccggaagaaattgcttatcgtaaagggtttattgatgctgagcaggtaaaagtattagccgaaccgttgaagaaaaatgcttatggtcagtatctgctcaaaatgattaaaggttattaataagatgaacgtaattaaaactgaaattcctgatgtgctgatttttgaaccaaaagtttttggggatgaacgtggcttcttttttgagagttttaatcagaggatttttgaagaagcagtaggtcgtaaggttgagtttgttcaggataaccattctaagtccagtaaaggtgttttacgtggtcttcattatcagttagaaccttatgctcaaggaaaactggtgcgctgtgttgttggcgaggtttttgatgttgcggttgatattcgtaaatcgtcacctacatttgggaaatgggttggggtgaatttgtctgctgagaataagcgtcagttgtggattcctgagggatttgcacatggttttttggtgctgagtgatttagcagaagttttatataaaacgaatcaatattatgctccatcacatgaaaaaaatattatatggaatgacctcttgcttaatattaaatggccgagcacagcactgatcactctgtctgataaggatgcaaatggggaaagatttgaactaagtgagttttgaaatgtctctcttaaaacatagtatatggaatgttgcgggctactttataccaacattaattgcaattcccgcctttggattaattgcgaggaaaattggtgtagaactatttggtttgtatacgttagcaatgatttttatagggtatgcaagtatatttgatgctgggttaacaagagctgttgtgcgtgaaatagcattactaaaaaacagagtggacgattgtaatacgataatagtaacttctattatcgctgtgatatttttagggtttatcggaggcgggggagtgtttctgcttaaaggcgatattattgaactgttaaatatctcaccaatatattacgccgattcgataaagtctctagtattattatcatctctgatacctgtattcttagtcacgcaaatactattagcagagcttgagggtcgggaatattttgggattctaaatatacaaaaaagtgtagggaattctttaattgcagggttacctgcattatttgttttaattaatcaaacgcttttttctgcaattattggtgtagcgattgcaagagttatatgcttgtggttaagctacattatgagcagggaaagaataactatcgatatctcatttttttcaataactgttttaaagcggttatttagatatggcgggtgggtaactataagtaacataatatctcctatattagcgagtatggatagatttattctatcccatatccagggagcatcaaaaatatcattctatacagtccctaatgagctggtaactaggcttggaatagttccaggctctcttgggaaagctgtttttccaaaattaagtcatgcaaggaattttacagcgtcatatgcagagcaaaaaaaagcttatatattaatgactgtcattgtaatgcctttggttttatttgtatattattacgcaaagtttattttaacattgtggatgggggctgagtatgcagggatttcggtcgaaatattacggattatgcttatagggtatatttttaactgttattcacaaatctcttttgccaacatacaggcctttggaaaagcaaaatacactgcatacatccatatgatggaatttattccttatttgataatgttatatataatttcaaaggaatatggggttattggtgttgcgtggttatggacaattcgagtaataattgattttttgatgcttttatatatgagttatcgttgtaataatcttatgaaaaaagggtagcctgatgatatatattgtggtattaaattggaatggggctatagataccattaattgtgttaaaagtttaatggatttaaatgttagcgattataaaattatcattgttgataactgttctatggataactcatatgatactataaaagaaaatcttaattcattatatattgctgataaaagtatcattgaggtgaagtatgaggatagaaataaatataaaaccttagaaaacgataaaatcatattaatacaatctccgcaaaataatgggtacgcaagtggtaataatattggcatagagttcgctcttaatcaggagaatatgaaatacgtctgggttctgaataatgatactgaagtggataaagaggctttaactcatttaattagtaaatgtgattcagataaaagtatagggatttgcggttctcgtttagtctattttgccgacagagagatgcagcaaggactaggtggggtgcataacaaatggttatgcactacaaaaaattatgaaatgggaagattagtttccaaaaaatatgatgatgaagtcattagtaatgatatagattatataattggcgcatcgatgtttttctctagagaatgtttggaaacagttggattgatgaatgaagaatattttttatactatgaagagttagatatttgcctcagagcaaaagcaaagaactttaaattaggtatttgctcagaaagtttggtttatcataaaataggtgcaagtactgatgggggaaagagcatgatggctgatctttgctcaataaaaaataggctggtcattacagaaaggttttatccccaatattattggacggtatggttgtcactttttgttgtagcatttaaccgtgctagaagaggtgagtttaataagatgaaaagatgtttgaatgttatgtttaacttcaaacgaaacaaaggtagcaaatgccattagaatatgcacttaatcatggtgttaataaatctatagtttgatatgttattaaagggtatttaatgaaagtggcttttttatctgcttatgatccactatctacatccagttggtctggcacaccttattatatgctaaaggcattatcgaagagaaatatttccattgaaatattaggaccggtaaatagctatatgatatacatgttaaaagtatataaattaatattaaggtgtttcggaaaagaatatgattatagtcattcgaagttgctttccaggtattacggtagaatattcggtaggaaattaaaaaaaattgatggtttggattttattatcgcacctgcaggttcctcacaaattgcttttttaaaaacaaccataccaataatatatctatcggatacaacatatgatcaattaaaaagctattatccgaatttaaataaaaaaacaattataaatgatgaggatgcaagtttaatcgaacgcaaggctattgaaaaagcaacagtagtatctttcccatctaaatgggcaatggatttttgcaggaattattacagattagattttgataaattagttgaaataccatggggggctaatttatttgatgatattcactttgctaataaaaatataattcaaaagaatagttatacttgtcttttcttgggagttgattgggaaagaaaaggtgggaaaacagccttgaaagcaattgaatatgtaaggcagttatatgggatcgatgttagactaaaaatttgtggatgtactccgaatcaaaagattttacctacttgggttgaattaattgataaagtagataaaaataacgttgacgaatatcagaaattcatcgatgtgttatctaacgctgatatacttcttttaccaaccattgctgaatgttatggaatggtattttgtgaagctgctgcttttggattgcctgttgtcgctacagatacaggtggagtcagttctatagttatcaacgaaaggacggggatattaattaaagacccgttagactataagcactttggaaatgcaattcataaaataattagttccgtagagacttatcaaaactactcccaaaacgcaagaattagatataataatatattgcattgggacaattgggctaaaaagataattgagattatgtatgagcataagaatagaagaatcaaatagcacaaaaagaattatatgtttatttatactttttcttgttttccctgattttttgttttatacattaggggttgataattttagcatttcaacgataatctcaattacattgctttttgtttttttaagagctaaaaatatttgcaaagataattttctaataatagtagcgttattcatattgttgtgttttaactgtttgttaagtatgctatttaatattgaacaggctttaacatttaaagttgtactttcaatatatagcatcttaataatggcatacgtctcctcttgttatgcacagacgttgtggttatgttctgaagaaatacttaagagatccgtcttttatttgttcgcatttctttgccttattggcattataagtattcttttacagaagactgagattatacatgataaaagtatgattctttttcctgaaccatcagcatttgcattggtttttatacctatcttttcattttgtttatactatacaagagggggggggctactattgctctatatattatctttgggtattgcgttaggtatccagaatttaacaatgttggtaggcattgtgattagtgtttttgtgatgaaaaaaataactataaggcaaactattgttatacttttgggggcatggattttttccatgatattaagtgatttagacatttcttactatacatcgcggcttgattttaaaaatactacgaacctatcagtgcttgtatatctttcaggaattgaaagagctttcttgaattttattacaagttatggtcttggtattggttttcaacaaatgggagtgaatggggagataggaatatatcaacaaattttagctgaacttgatgcccctatgttaaatatatacgatggctcatttatttcttctaagttaatatctgagtttggggttattggtgcattaatgtgtattttctattttttttatttttcccgattttatctgcgtttcaaaaaaagtaagagatattcaccgcagtatattttagcatatagcttctacatgtgtttcttcatccctctttttatacgtggtgctggttatataaacccctatgtgtttatgttattttcatcaatatttttgtgcaaatatcacgctaaaaatatcttgatgaaatctaatgtccagatagctatataatagtagattatattatcattatcacgtaaattacatattaatagcatatatgataactaggacataaataatgtgcattaaaaaaaaacttaagttaattaaacgatatggcctttatggtggtcttaggcttcttaaagatatattcttaacaaaatttttattttgttcaaatgttaggattattagatttccatgttatattagaaaagatggaagtgttagttttggaaaaggttttacatcaggtgtaggattacgagttgatgcatttatggatgccgtagtttccattggagaaaatgttcaaattaatgactatgttcacatcgcggctattaataatgtcattattggtagagatacattaatagcaagtaaagtatttattagtgatcataatcatggtattttttctaaatccgatatccatagttcaccaactattattccttcgtctaggccccttgaatctgcacctgtgtatattggagagcgtgtgtggattggcgaaaatgtgacaatattaccaggtgcgtgtataggtaatggtgtagttattggcgcaaacagtgttgttcgtggtgagattcctaataatgtgatcattgctggtgttccagctaaaattgttaaaaaatataactatgagcgtatgcaatgggaaagaatatagttgtaatatcggctgttaattttacaaccggaggcccctttaccgtactaaaaaatgtgcttacagcaactaaagatagagccgaatgtaaatttattgcactggttcatagctctgctgaactaatggaattatttccgtgggttgaatttatagagtatccagaagtcaagtcttcgtgggttaaaagattatatttcgaatatataacttgcaatagattatctaaggtgattaaggcaactcattgggtatgcttacatgatattacagcaaatgttagtgtaccctatagatttgtttattgccacaatcctgcaccgttctataaatatttaagctatcgagatattataggagaacctaaattttatcttttttatcttttttatgggcttttatacaatatcaatataaaaaagaacacagcagtttttgttcagcagcagtggctaaaaaaagaattcgaaaaaaaatataagttaaagaatgttgttgttagtcgccctgaagatatttgcccttttgaaagtgatggtttggtaagaaataataataaaaaggatgtgaggatattttacccagcagtgccccgtatatttaaaaactttgaagttatcatacgtgctgcacaaatattacaagataaaaatattcatttttatcttacttttgatggtactgaaaataagtatgcaaaaagaatatataaattagcttccgaactgaaaaatgtacatttcctcggttaccttaatgcaaccgagatggttaacttttatcaagattcagatattatttgtttcccatcgaaactagaaacgtggggattaccattatcagaagctaaaacatacaaaaaatggatatttgcggcagacttaccttatgctcatgaagttttatataactattcaaaaactagatattttccatttgacgatgagaaaatacttgttcgctacatattagagtacacaagtaaaaatatgcatgaagatataaaaaatagtagggtgaattttaataatgatgcattgactggttttgaacagtttattgaatatatcctcaaggggaactgacgtggtttatattataatcgtttcacatggccatgatgactatatagaaaatcttttattaaatttaaagttgccctctggaagatttaaaataatagttcgtgataacaaaagttcaatggttttaaaaaaaacatgcgaaaaaaattgcgtaacctatttgcatggagggcaatatggatttggacataataataacatagcagtgtcatatataattaataacttcatgattatgaataatgattattttctctttcttaaccccgatgtattcataaccagtgaaagtttgattaattatgttgattatataattagtaatgattataagtttagcacattatgtctttatcgagattttactaaaagcaaacatgattattcaatacggagttttccaactttatatgattttctttgttcttttttattgggggtgaataaaagtaaaattaagaaggaaaatatactttctgatactgtagttgattggtgtgctggctcatttatgcttattcatgctttaagtttcttaaatgtgaatggttttgatcaaaaatattttatgtattgtgaagatattgacctttgtatgcgtttaaaattaagtggagtagatctttactatactccccattttgatgctattcattatgcgcagcatgaaaatagaagaatatttactaaagcatttcgatggcatataaggagtattacgcgctacatattacggaaaccaattctttcttataaaaactatagaaaaattacatccgaactggtaaagtga

SEQ ID NO: 13 - protein, 652 aa, Artificial Sequence
  Detoxified EPA protein comprising 4 optimized N-glycosylation sequences
GSGGGDQNATGSGGGKLAEEAFDLWNECAKACVLDLKDGVRSSRMSVDPAIADTNGQGVLHYSMVLEGGNDALKLAIDNALSITSDGLTIRLEGGVEPNKPVRYSYTRQARGSWSLNWLVPIGHEKPSNIKVFIHELNAGNQLSHMSPIYTIEMGDELLAKLARDATFFVRAHESNEMQPTLAISHAGVSVVMAQAQPRREKRWSEWASGKVLCLLDPLDGVYNYLAQQRCNLDDTWEGKIYRVLAGNPAKHDLDIKDNNNSTPTVISHRLHFPEGGSLAALTAHQACHLPLEAFTRHRQPRGWEQLEQCGYPVQRLVALYLAARLSWNQVDQVIRNALASPGSGGDLGEAIREQPEQARLALTLAAAESERFVRQGTGNDEAGAASADVVSLTCPVAKDQNRTKGECAGPADSGDALLERNYPTGAEFLGDGGDVSFSTRGTQNWTVERLLQAHRQLEERGYVFVGYHGTFLEAAQSIVFGGVRARSQDLDAIWRGFYIAGDPALAYGYAQDQEPDARGRIRNGALLRVYVPRWSLPGFYRTGLTLAAPEAAGEVERLIGHPLPLRLDAITGPEEEGGRVTILGWPLAERTVVIPSAIPTDPRNVGGDLDPSSIPDKEQAISALPDYASQPGKPPREDLKLGSGGGDQNAT

SEQ ID NO: 14 - protein, 3 aa, Artificial Sequence
  N-glycosylation consensus sequence
  VARIANT (2)..(2): Xaa = any amino acid
  VARIANT (3)..(3): Xaa = Ser or Thr
NXX

SEQ ID NO: 15 - protein, 5 aa, Artificial Sequence
  N-glycosylation consensus sequence
  VARIANT (1)..(1): Xaa = Asp or Glu
  VARIANT (2)..(2): Xaa = independently selected from any natural amino acid except Pro
  VARIANT (4)..(4): Xaa = independently selected from any natural amino acid except Pro
  VARIANT (5)..(5): Xaa = Ser or Thr
XXNXX